European Patent Application EP 4 410 809 A1, published August 7, 2024. Title: PEPTIDE HAVING ANTI-AGING ACTIVITY, AND USE THEREOF. Applicant: CAREGEN CO., LTD. Application KR. The sequence listing filed with the application follows.

SEQUENCE LISTING (13 sequences)

SEQ ID NO: 1 - protein, 10 aa, synthetic construct
  REGION 1..10: note = peptide
EYIPNRVCRR

SEQ ID NO: 2 - DNA, 20 bp, synthetic construct
  misc_feature 1..20: note = Col1a1-F
  source 1..20: mol_type = other DNA
caccctcaagagcctgagtc

SEQ ID NO: 3 - DNA, 20 bp, synthetic construct
  misc_feature 1..20: note = Col1a1-R
  source 1..20: mol_type = other DNA
agacggctgagtagggaaca

SEQ ID NO: 4 - DNA, 20 bp, synthetic construct
  misc_feature 1..20: note = Fibronectin-F
  source 1..20: mol_type = other DNA
ccaggaaccgagtacaccat

SEQ ID NO: 5 - DNA, 20 bp, synthetic construct
  misc_feature 1..20: note = Fibronectin-R
  source 1..20: mol_type = other DNA
atacccaggttgggtgatga

SEQ ID NO: 6 - DNA, 20 bp, synthetic construct
  misc_feature 1..20: note = Elastin-F
  source 1..20: mol_type = other DNA
gcaagacctggctttggact

SEQ ID NO: 7 - DNA, 21 bp, synthetic construct
  misc_feature 1..21: note = Elastin-R
  source 1..21: mol_type = other DNA
gggagtttctggttagggctg

SEQ ID NO: 8 - DNA, 20 bp, synthetic construct
  misc_feature 1..20: note = GAPDH-F
  source 1..20: mol_type = other DNA
ggagccaaaagggtcatcat

SEQ ID NO: 9 - DNA, 20 bp, synthetic construct
  misc_feature 1..20: note = GAPDH-R
  source 1..20: mol_type = other DNA
gtgatggcatggactgtggt

SEQ ID NO: 10 - DNA, 20 bp, synthetic construct
  misc_feature 1..20: note = SIRT1-F
  source 1..20: mol_type = other DNA
tcagtggctggaacagtgag

SEQ ID NO: 11 - DNA, 20 bp, synthetic construct
  misc_feature 1..20: note = SIRT1-R
  source 1..20: mol_type = other DNA
tctggcatgtcccactatca

SEQ ID NO: 12 - DNA, 20 bp, synthetic construct
  misc_feature 1..20: note = AQP3-F
  source 1..20: mol_type = other DNA
ccttcttgggtgctggaata

SEQ ID NO: 13 - DNA, 20 bp, synthetic construct
  misc_feature 1..20: note = AQP3-R
  source 1..20: mol_type = other DNA
acacgataagggaggctgtg